European Patent Application EP 4 410 960 A1, published August 7, 2024. Title: Inducer of Viral Vector Production. Applicant: 株式会社カネカ. The sequence listing filed with the application follows.

SEQUENCE LISTING (18 sequences)

SEQ ID NO: 1 - DNA, 20 bp, synthetic construct
  misc_feature 1..20: note = Primer Fw
  source 1..20: mol_type = other DNA
tgggttcaagcgattctcct

SEQ ID NO: 2 - DNA, 21 bp, synthetic construct
  misc_feature 1..21: note = Primer Re
  source 1..21: mol_type = other DNA
cctgtaatcccagcaatttgg

SEQ ID NO: 3 - DNA, 720 bp, synthetic construct
  misc_feature 1..720: note = Venus
  source 1..720: mol_type = other DNA
atggtgagcaagggcgaggagctgttcaccggggtggtgcccatcctggtcgagctggacggcgacgtaaacggccacaagttcagcgtgtccggcgagggcgagggcgatgccacctacggcaagctgaccctgaagctgatctgcaccaccggcaagctgcccgtgccctggcccaccctcgtgaccaccctgggctacggcctgcagtgcttcgcccgctaccccgaccacatgaagcagcacgacttcttcaagtccgccatgcccgaaggctacgtccaggagcgcaccatcttcttcaaggacgacggcaactacaagacccgcgccgaggtgaagttcgagggcgacaccctggtgaaccgcatcgagctgaagggcatcgacttcaaggaggacggcaacatcctggggcacaagctggagtacaactacaacagccacaacgtctatatcaccgccgacaagcagaagaacggcatcaaggccaacttcaagatccgccacaacatcgaggacggcggcgtgcagctcgccgaccactaccagcagaacacccccatcggcgacggccccgtgctgctgcccgacaaccactacctgagctaccagtccgccctgagcaaagaccccaacgagaagcgcgatcacatggtcctgctggagttcgtgaccgccgccgggatcactctcggcatggacgagctgtacaagtaa

SEQ ID NO: 4 - DNA, 1896 bp, Escherichia virus N15
  misc_feature 1..1896: note = TelN
  source 1..1896: mol_type = genomic DNA
atgagcaaggtaaaaatcggtgagttgatcaacacgcttgtgaatgaggtagaggcaattgatgcctcagaccgcccacaaggcgacaaaacgaagagaattaaagccgcagccgcacggtataagaacgcgttatttaatgataaaagaaagttccgtgggaaaggattgcagaaaagaataaccgcgaatacttttaacgcctatatgagcagggcaagaaagcggtttgatgataaattacatcatagctttgataaaaatattaataaattatcggaaaagtatcctctttacagcgaagaattatcttcatggctttctatgcctacggctaatattcgccagcacatgtcatcgttacaatctaaattgaaagaaataatgccgcttgccgaagagttatcaaatgtaagaataggctctaaaggcagtgatgcaaaaatagcaagactaataaaaaaatatccagattggagttttgctcttagtgatttaaacagtgatgattggaaggagcgccgtgactatctttataagttattccaacaaggctctgcgttgttagaagaactacaccagctcaaggtcaaccatgaggttctgtaccatctgcagctaagccctgcggagcgtacatctatacagcaacgatgggccgatgttctgcgcgagaagaagcgtaatgttgtggttattgactacccaacatacatgcagtctatctatgatattttgaataatcctgcgactttatttagtttaaacactcgttctggaatggcacctttggcctttgctctggctgcggtatcagggcgaagaatgattgagataatgtttcagggtgaatttgccgtttcaggaaagtatacggttaatttctcagggcaagctaaaaaacgctctgaagataaaagcgtaaccagaacgatttatactttatgcgaagcaaaattattcgttgaattattaacagaattgcgttcttgctctgctgcatctgatttcgatgaggttgttaaaggatatggaaaggatgatacaaggtctgagaacggcaggataaatgctattttagcaaaagcatttaacccttgggttaaatcatttttcggcgatgaccgtcgtgtttataaagatagccgcgctatttacgctcgcatcgcttatgagatgttcttccgcgtcgatccacggtggaaaaacgtcgacgaggatgtgttcttcatggagattctcggacacgacgatgagaacacccagctgcactataagcagttcaagctggccaacttctccagaacctggcgacctgaagttggggatgaaaacaccaggctggtggctctgcagaaactggacgatgaaatgccaggctttgccagaggtgacgctggcgtccgtctccatgaaaccgttaagcagctggtggagcaggacccatcagcaaaaataaccaacagcactctccgggcctttaaatttagcccgacgatgattagccggtacctggagtttgccgctgatgcattggggcagttcgttggcgagaacgggcagtggcagctgaagatagagacacctgcaatcgtcctgcctgatgaagaatccgttgagaccatcgacgaaccggatgatgagtcccaagacgacgagctggatgaagatgaaattgagctcgacgagggtggcggcgatgaaccaaccgaagaggaagggccagaagaacatcagccaactgctctaaaacccgtcttcaagcctgcaaaaaataacggggacggaacgtacaagatagagtttgaatacgatggaaagcattatgcctggtccggccccgccgatagccctatggccgcaatgcgatccgcatgggaaacgtactacagctaa

SEQ ID NO: 5 - DNA, 56 bp, synthetic construct
  misc_feature 1..56: note = telRL
  source 1..56: mol_type = other DNA
tatcagcacacaattgcccattatacgcgcgtataatggactattgtgtgctgata

SEQ ID NO: 6 - DNA, 1143 bp, synthetic construct
  misc_feature 1..1143: note = AraC
  source 1..1143: mol_type = other DNA
gctaatcttatggataaaaatgctatggcatagcaaagtgtgacgccgtgcaaataatcaatgtggacttttctgccgtgattatagacacttttgttacgcgtttttgtcatggctttggtcccgctttgttacagaatgcttttaataagcggggttaccggtttggttagcgagaagagccagtaaaagacgcagtgacggcaatgtctgatgcaatatggacaattggtttcttctctgaatggcgggagtatgaaaagtatggctgaagcgcaaaatgatcccctgctgccgggatactcgtttaatgcccatctggtggcgggtttaacgccgattgaggccaacggttatctcgatttttttatcgaccgaccgctgggaatgaaaggttatattctcaatctcaccattcgcggtcagggggtggtgaaaaatcagggacgagaatttgtttgccgaccgggtgatattttgctgttcccgccaggagagattcatcactacggtcgtcatccggaggctcgcgaatggtatcaccagtgggtttactttcgtccgcgcgcctactggcatgaatggcttaactggccgtcaatatttgccaatacggggttctttcgcccggatgaagcgcaccagccgcatttcagcgacctgtttgggcaaatcattaacgccgggcaaggggaagggcgctattcggagctgctggcgataaatctgcttgagcaattgttactgcggcgcatggaagcgattaacgagtcgctccatccaccgatggataatcgggtacgcgaggcttgtcagtacatcagcgatcacctggcagacagcaattttgatatcgccagcgtcgcacagcatgtttgcttgtcgccgtcgcgtctgtcacatcttttccgccagcagttagggattagcgtcttaagctggcgcgaggaccaacgtatcagccaggcgaagctgcttttgagcaccacccggatgcctatcgccaccgtcggtcgcaatgttggttttgacgatcaactctatttctcgcgggtatttaaaaaatgcaccggggccagcccgagcgagttccgtgccggttgtgaagaaaaagtgaatgatgtagccgtcaagttgtcataa

SEQ ID NO: 7 - DNA, 55 bp, synthetic construct
  misc_feature 1..55: note = promoter
  source 1..55: mol_type = other DNA
tacctgacgctttttatcgcaactctctactgtttctccatacccgtttttttgg

SEQ ID NO: 8 - DNA, 24 bp, synthetic construct
  misc_feature 1..24: note = TelN Fw
  source 1..24: mol_type = other DNA
atgagcaaggtaaaaatcggtgag

SEQ ID NO: 9 - DNA, 23 bp, synthetic construct
  misc_feature 1..23: note = TelN Re
  source 1..23: mol_type = other DNA
ttagctgtagtacgtttcccatg

SEQ ID NO: 10 - DNA, 27 bp, synthetic construct
  misc_feature 1..27: note = AraC Fw
  source 1..27: mol_type = other DNA
gctaatcttatggataaaaatgctatg

SEQ ID NO: 11 - DNA, 24 bp, synthetic construct
  misc_feature 1..24: note = AraC Re
  source 1..24: mol_type = other DNA
ttatgacaacttgacggctacatc

SEQ ID NO: 12 - DNA, 19 bp, synthetic construct
  misc_feature 1..19: note = Venus Fw
  source 1..19: mol_type = other DNA
atggtgagcaagggcgagg

SEQ ID NO: 13 - DNA, 22 bp, synthetic construct
  misc_feature 1..22: note = Venus Re
  source 1..22: mol_type = other DNA
ttacttgtacagctcgtccatg

SEQ ID NO: 14 - DNA, 1866 bp, Adeno associated virus
  misc_feature 1..1866: note = Rep
  source 1..1866: mol_type = genomic DNA
atgccggggttttacgagattgtgattaaggtccccagcgaccttgacgagcatctgcccggcatttctgacagctttgtgaactgggtggccgagaaggaatgggagttgccgccagattctgacatggatctgaatctgattgagcaggcacccctgaccgtggccgagaagctgcagcgcgactttctgacggaatggcgccgtgtgagtaaggccccggaggcccttttctttgtgcaatttgagaagggagagagctacttccacatgcacgtgctcgtggaaaccaccggggtgaaatccatggttttgggacgtttcctgagtcagattcgcgaaaaactgattcagagaatttaccgcgggatcgagccgactttgccaaactggttcgcggtcacaaagaccagaaatggcgccggaggcgggaacaaggtggtggatgagtgctacatccccaattacttgctccccaaaacccagcctgagctccagtgggcgtggactaatatggaacagtatttaagcgcctgtttgaatctcacggagcgtaaacggttggtggcgcagcatctgacgcacgtgtcgcagacgcaggagcagaacaaagagaatcagaatcccaattctgatgcgccggtgatcagatcaaaaacttcagccaggtacatggagctggtcgggtggctcgtggacaaggggattacctcggagaagcagtggatccaggaggaccaggcctcatacatctccttcaatgcggcctccaactcgcggtcccaaatcaaggctgccttggacaatgcgggaaagattatgagcctgactaaaaccgcccccgactacctggtgggccagcagcccgtggaggacatttccagcaatcggatttataaaattttggaactaaacgggtacgatccccaatatgcggcttccgtctttctgggatgggccacgaaaaagttcggcaagaggaacaccatctggctgtttgggcctgcaactaccgggaagaccaacatcgcggaggccatagcccacactgtgcccttctacgggtgcgtaaactggaccaatgagaactttcccttcaacgactgtgtcgacaagatggtgatctggtgggaggaggggaagatgaccgccaaggtcgtggagtcggccaaagccattctcggaggaagcaaggtgcgcgtggaccagaaatgcaagtcctcggcccagatagacccgactcccgtgatcgtcacctccaacaccaacatgtgcgccgtgattgacgggaactcaacgaccttcgaacaccagcagccgttgcaagaccggatgttcaaatttgaactcacccgccgtctggatcatgactttgggaaggtcaccaagcaggaagtcaaagactttttccggtgggcaaaggatcacgtggttgaggtggagcatgaattctacgtcaaaaagggtggagccaagaaaagacccgcccccagtgacgcagatataagtgagcccaaacgggtgcgcgagtcagttgcgcagccatcgacgtcagacgcggaagcttcgatcaactacgcagacaggtaccaaaacaaatgttctcgtcacgtgggcatgaatctgatgctgtttccctgcagacaatgcgagagaatgaatcagaattcaaatatctgcttcactcacggacagaaagactgtttagagtgctttcccgtgtcagaatctcaacccgtttctgtcgtcaaaaaggcgtatcagaaactgtgctacattcatcatatcatgggaaaggtgccagacgcttgcactgcctgcgatctggtcaatgtggatttggatgactgcatctttgaacaataa

SEQ ID NO: 15 - DNA, 2208 bp, Adeno associated virus
  misc_feature 1..2208: note = Cap
  source 1..2208: mol_type = genomic DNA
atggctgccgatggttatcttccagattggctcgaggacactctctctgaaggaataagacagtggtggaagctcaaacctggcccaccaccaccaaagcccgcagagcggcataaggacgacagcaggggtcttgtgcttcctgggtacaagtacctcggacccttcaacggactcgacaagggagagccggtcaacgaggcagacgccgcggccctcgagcacgacaaagcctacgaccggcagctcgacagcggagacaacccgtacctcaagtacaaccacgccgacgcggagtttcaggagcgccttaaagaagatacgtcttttgggggcaacctcggacgagcagtcttccaggcgaaaaagagggttcttgaacctctgggcctggttgaggaacctgttaagacggctccgggaaaaaagaggccggtagagcactctcctgtggagccagactcctcctcgggaaccggaaaggcgggccagcagcctgcaagaaaaagattgaattttggtcagactggagacgcagactcagtacctgacccccagcctctcggacagccaccagcagccccctctggtctgggaactaatacgatggctacaggcagtggcgcaccaatggcagacaataacgagggcgccgacggagtgggtaattcctcgggaaattggcattgcgattccacatggatgggcgacagagtcatcaccaccagcacccgaacctgggccctgcccacctacaacaaccacctctacaaacaaatttccagccaatcaggagcctcgaacgacaatcactactttggctacagcaccccttgggggtattttgacttcaacagattccactgccacttttcaccacgtgactggcaaagactcatcaacaacaactggggattccgacccaagagactcaacttcaagctctttaacattcaagtcaaagaggtcacgcagaatgacggtacgacgacgattgccaataaccttaccagcacggttcaggtgtttactgactcggagtaccagctcccgtacgtcctcggctcggcgcatcaaggatgcctcccgccgttcccagcagacgtcttcatggtgccacagtatggatacctcaccctgaacaacgggagtcaggcagtaggacgctcttcattttactgcctggagtactttccttctcagatgctgcgtaccggaaacaactttaccttcagctacacttttgaggacgttcctttccacagcagctacgctcacagccagagtctggaccgtctcatgaatcctctcatcgaccagtacctgtattacttgagcagaacaaacactccaagtggaaccaccacgcagtcaaggcttcagttttctcaggccggagcgagtgacattcgggaccagtctaggaactggcttcctggaccctgttaccgccagcagcgagtatcaaagacatctgcggataacaacaacagtgaatactcgtggactggagctaccaagtaccacctcaatggcagagactctctggtgaatccgggcccggccatggcaagccacaaggacgatgaagaaaagttttttcctcagagcggggttctcatctttgggaagcaaggctcagagaaaacaaatgtggacattgaaaaggtcatgattacagacgaagaggaaatcaggacaaccaatcccgtggctacggagcagtatggttctgtatctaccaacctccagagaggcaacagacaagcagctaccgcagatgtcaacacacaaggcgttcttccaggcatggtctggcaggacagagatgtgtaccttcaggggcccatctgggcaaagattccacacacggacggacattttcacccctctcccctcatgggtggattcggacttaaacaccctcctccacagattctcatcaagaacaccccggtacctgcgaatccttcgaccaccttcagtgcggcaaagtttgcttccttcatcacacagtactccacgggacaggtcagcgtggagatcgagtgggagctgcagaaggaaaacagcaaacgctggaatcccgaaattcagtacacttccaactacaacaagtctgttaatgtggactttactgtggacactaatggcgtgtattcagagcctcgccccattggcaccagatacctgactcgtaatctgtaa

SEQ ID NO: 16 - DNA, 5336 bp, Adenovirus
  misc_feature 1..5336: note = E2A
  source 1..5336: mol_type = genomic DNA
ggtacccaactccatgcttaacagtccccaggtacagcccaccctgcgtcgcaaccaggaacagctctacagcttcctggagcgccactcgccctacttccgcagccacagtgcgcagattaggagcgccacttctttttgtcacttgaaaaacatgtaaaaataatgtactaggagacactttcaataaaggcaaatgtttttatttgtacactctcgggtgattatttaccccccacccttgccgtctgcgccgtttaaaaatcaaaggggttctgccgcgcatcgctatgcgccactggcagggacacgttgcgatactggtgtttagtgctccacttaaactcaggcacaaccatccgcggcagctcggtgaagttttcactccacaggctgcgcaccatcaccaacgcgtttagcaggtcgggcgccgatatcttgaagtcgcagttggggcctccgccctgcgcgcgcgagttgcgatacacagggttgcagcactggaacactatcagcgccgggtggtgcacgctggccagcacgctcttgtcggagatcagatccgcgtccaggtcctccgcgttgctcagggcgaacggagtcaactttggtagctgccttcccaaaaagggtgcatgcccaggctttgagttgcactcgcaccgtagtggcatcagaaggtgaccgtgcccggtctgggcgttaggatacagcgcctgcatgaaagccttgatctgcttaaaagccacctgagcctttgcgccttcagagaagaacatgccgcaagacttgccggaaaactgattggccggacaggccgcgtcatgcacgcagcaccttgcgtcggtgttggagatctgcaccacatttcggccccaccggttcttcacgatcttggccttgctagactgctccttcagcgcgcgctgcccgttttcgctcgtcacatccatttcaatcacgtgctccttatttatcataatgctcccgtgtagacacttaagctcgccttcgatctcagcgcagcggtgcagccacaacgcgcagcccgtgggctcgtggtgcttgtaggttacctctgcaaacgactgcaggtacgcctgcaggaatcgccccatcatcgtcacaaaggtcttgttgctggtgaaggtcagctgcaacccgcggtgctcctcgtttagccaggtcttgcatacggccgccagagcttccacttggtcaggcagtagcttgaagtttgcctttagatcgttatccacgtggtacttgtccatcaacgcgcgcgcagcctccatgcccttctcccacgcagacacgatcggcaggctcagcgggtttatcaccgtgctttcactttccgcttcactggactcttccttttcctcttgcgtccgcataccccgcgccactgggtcgtcttcattcagccgccgcaccgtgcgcttacctcccttgccgtgcttgattagcaccggtgggttgctgaaacccaccatttgtagcgccacatcttctctttcttcctcgctgtccacgatcacctctggggatggcgggcgctcgggcttgggagaggggcgcttctttttctttttggacgcaatggccaaatccgccgtcgaggtcgatggccgcgggctgggtgtgcgcggcaccagcgcatcttgtgacgagtcttcttcgtcctcggactcgagacgccgcctcagccgcttttttgggggcgcgcggggaggcggcggcgacggcgacggggacgacacgtcctccatggttggtggacgtcgcgccgcaccgcgtccgcgctcgggggtggtttcgcgctgctcctcttcccgactggccatttccttctcctataggcagaaaaagatcatggagtcagtcgagaaggaggacagcctaaccgccccctttgagttcgccaccaccgcctccaccgatgccgccaacgcgcctaccaccttccccgtcgaggcacccccgcttgaggaggaggaagtgattatcgagcaggacccaggttttgtaagcgaagacgacgaggatcgctcagtaccaacagaggataaaaagcaagaccaggacgacgcagaggcaaacgaggaacaagtcgggcggggggaccaaaggcatggcgactacctagatgtgggagacgacgtgctgttgaagcatctgcagcgccagtgcgccattatctgcgacgcgttgcaagagcgcagcgatgtgcccctcgccatagcggatgtcagccttgcctacgaacgccacctgttctcaccgcgcgtaccccccaaacgccaagaaaacggcacatgcgagcccaacccgcgcctcaacttctaccccgtatttgccgtgccagaggtgcttgccacctatcacatctttttccaaaactgcaagatacccctatcctgccgtgccaaccgcagccgagcggacaagcagctggccttgcggcagggcgctgtcatacctgatatcgcctcgctcgacgaagtgccaaaaatctttgagggtcttggacgcgacgagaaacgcgcggcaaacgctctgcaacaagaaaacagcgaaaatgaaagtcactgtggagtgctggtggaacttgagggtgacaacgcgcgcctagccgtgctgaaacgcagcatcgaggtcacccactttgcctacccggcacttaacctaccccccaaggttatgagcacagtcatgagcgagctgatcgtgcgccgtgcacgacccctggagagggatgcaaacttgcaagaacaaaccgaggagggcctacccgcagttggcgatgagcagctggcgcgctggcttgagacgcgcgagcctgccgacttggaggagcgacgcaagctaatgatggccgcagtgcttgttaccgtggagcttgagtgcatgcagcggttctttgctgacccggagatgcagcgcaagctagaggaaacgttgcactacacctttcgccagggctacgtgcgccaggcctgcaaaatttccaacgtggagctctgcaacctggtctcctaccttggaattttgcacgaaaaccgcctcgggcaaaacgtgcttcattccacgctcaagggcgaggcgcgccgcgactacgtccgcgactgcgtttacttatttctgtgctacacctggcaaacggccatgggcgtgtggcagcaatgcctggaggagcgcaacctaaaggagctgcagaagctgctaaagcaaaacttgaaggacctatggacggccttcaacgagcgctccgtggccgcgcacctggcggacattatcttccccgaacgcctgcttaaaaccctgcaacagggtctgccagacttcaccagtcaaagcatgttgcaaaactttaggaactttatcctagagcgttcaggaattctgcccgccacctgctgtgcgcttcctagcgactttgtgcccattaagtaccgtgaatgccctccgccgctttggggtcactgctaccttctgcagctagccaactaccttgcctaccactccgacatcatggaagacgtgagcggtgacggcctactggagtgtcactgtcgctgcaacctatgcaccccgcaccgctccctggtctgcaattcgcaactgcttagcgaaagtcaaattatcggtacctttgagctgcagggtccctcgcctgacgaaaagtccgcggctccggggttgaaactcactccggggctgtggacgtcggcttaccttcgcaaatttgtacctgaggactaccacgcccacgagattaggttctacgaagaccaatcccgcccgccaaatgcggagcttaccgcctgcgtcattacccagggccacatccttggccaattgcaagccatcaacaaagcccgccaagagtttctgctacgaaagggacggggggtttacctggacccccagtccggcgaggagctcaacccaatccccccgccgccgcagccctatcagcagccgcgggcccttgcttcccaggatggcacccaaaaagaagctgcagctgccgccgccgccacccacggacgaggaggaatactgggacagtcaggcagaggaggttttggacgaggaggaggagatgatggaagactgggacagcctagacgaagcttccgaggccgaagaggtgtcagacgaaacaccgtcaccctcggtcgcattcccctcgccggcgccccagaaattggcaaccgttcccagcatcgctacaacctccgctcctcaggcgccgccggcactgcctgttcgccgacccaaccgtagatgggacaccactggaaccagggccggtaagtctaagcagccgccgccgttagcccaagagcaacaacagcgccaaggctaccgctcgtggcgcgggcacaagaacgccatagttgcttgcttgcaagactgtgggggcaacatctccttcgcccgccgctttcttctctaccatcacggcgtggccttcccccgtaacatcctgcattactaccgtcatctctacagcccctactgcaccggcggcagcggcagcggcagcaacagcagcggtcacacagaagcaaaggcgaccggatagcaagactctgacaaagcccaagaaatccacagcggcggcagcagcaggaggaggagcgctgcgtctggcgcccaacgaacccgtatcgacccgcgagcttagaaataggatttttcccactctgtatgctatatttcaacaaagcaggggccaagaacaagagctgaaaataaaaaacaggtctctgcgctccctcacccgcagctgcctgtatcacaaaagcgaagatcagcttcggcgcacgctggaagacgcggaggctctcttcagcaaatactgcgcgctgactcttaaggactagtttcgcgccctttctcaaatttaagcgcgaaaactacgtcatctccagcggccacacccggcgccagcacctgtcgtcagcgccattatgagcaaggaaattcccacgccctacatgtggagttaccagccacaaatgggacttgcggctggagctgcccaagactactcaacccgaataaactacatgagcgcgggaccccacatgatatcccgggtcaacggaatccgcgcccaccgaaaccgaattctcctcgaacaggcggctattaccaccacacctcgtaataaccttaatccccgtagttggcccgctgccctggtgtaccaggaaagtcccgctcccaccactgtggtacttcccagagacgcccaggccgaagttcagatgactaactcaggggcgcagcttgcgggcggctttcgtcacagggtgcggtcg

SEQ ID NO: 17 - DNA, 3201 bp, Adenovirus
  misc_feature 1..3201: note = E4
  source 1..3201: mol_type = genomic DNA
cccgggcgttttagggcggagtaacttgcatgtattgggaattgtagtttttttaaaatgggaagtgacgtatcgtgggaaaacggaagtgaagatttgaggaagttgtgggttttttggctttcgtttctgggcgtaggttcgcgtgcggttttctgggtgttttttgtggactttaaccgttacgtcattttttagtcctatatatactcgctctgtacttggccctttttacactgtgactgattgagctggtgccgtgtcgagtggtgttttttaataggtttttttactggtaaggctgactgttatggctgccgctgtggaagcgctgtatgttgttctggagcgggagggtgctattttgcctaggcaggagggtttttcaggtgtttatgtgtttttctctcctattaattttgttatacctcctatgggggctgtaatgttgtctctacgcctgcgggtatgtattcccccgggctatttcggtcgctttttagcactgaccgatgttaaccaacctgatgtgtttaccgagtcttacattatgactccggacatgaccgaggaactgtcggtggtgctttttaatcacggtgaccagtttttttacggtcacgccggcatggccgtagtccgtcttatgcttataagggttgtttttcctgttgtaagacaggcttctaatgtttaaatgtttttttttttgttattttattttgtgtttaatgcaggaacccgcagacatgtttgagagaaaaatggtgtctttttctgtggtggttccggaacttacctgcctttatctgcatgagcatgactacgatgtgcttgcttttttgcgcgaggctttgcctgattttttgagcagcaccttgcattttatatcgccgcccatgcaacaagcttacataggggctacgctggttagcatagctccgagtatgcgtgtcataatcagtgtgggttcttttgtcatggttcctggcggggaagtggccgcgctggtccgtgcagacctgcacgattatgttcagctggccctgcgaagggacctacgggatcgcggtatttttgttaatgttccgcttttgaatcttatacaggtctgtgaggaacctgaatttttgcaatcatgattcgctgcttgaggctgaaggtggagggcgctctggagcagatttttacaatggccggacttaatattcgggatttgcttagagacatattgataaggtggcgagatgaaaattatttgggcatggttgaaggtgctggaatgtttatagaggagattcaccctgaagggtttagcctttacgtccacttggacgtgagggcagtttgccttttggaagccattgtgcaacatcttacaaatgccattatctgttctttggctgtagagtttgaccacgccaccggaggggagcgcgttcacttaatagatcttcattttgaggttttggataatcttttggaataaaaaaaaaaaaacatggttcttccagctcttcccgctcctcccgtgtgtgactcgcagaacgaatgtgtaggttggctgggtgtggcttattctgcggtggtggatgttatcagggcagcggcgcatgaaggagtttacatagaacccgaagccagggggcgcctggatgctttgagagagtggatatactacaactactacacagagcgagctaagcgacgagaccggagacgcagatctgtttgtcacgcccgcacctggttttgcttcaggaaatatgactacgtccggcgttccatttggcatgacactacgaccaacacgatctcggttgtctcggcgcactccgtacagtagggatcgcctacctccttttgagacagagacccgcgctaccatactggaggatcatccgctgctgcccgaatgtaacactttgacaatgcacaacgtgagttacgtgcgaggtcttccctgcagtgtgggatttacgctgattcaggaatgggttgttccctgggatatggttctgacgcgggaggagcttgtaatcctgaggaagtgtatgcacgtgtgcctgtgttgtgccaacattgatatcatgacgagcatgatgatccatggttacgagtcctgggctctccactgtcattgttccagtcccggttccctgcagtgcatagccggcgggcaggttttggccagctggtttaggatggtggtggatggcgccatgtttaatcagaggtttatatggtaccgggaggtggtgaattacaacatgccaaaagaggtaatgtttatgtccagcgtgtttatgaggggtcgccacttaatctacctgcgcttgtggtatgatggccacgtgggttctgtggtccccgccatgagctttggatacagcgccttgcactgtgggattttgaacaatattgtggtgctgtgctgcagttactgtgctgatttaagtgagatcagggtgcgctgctgtgcccggaggacaaggcgtctcatgctgcgggcggtgcgaatcatcgctgaggagaccactgccatgttgtattcctgcaggacggagcggcggcggcagcagtttattcgcgcgctgctgcagcaccaccgccctatcctgatgcacgattatgactctacccccatgtaggcgtggacttccccttcgccgcccgttgagcaaccgcaagttggacagcagcctgtggctcagcagctggacagcgacatgaacttaagcgagctgcccggggagtttattaatatcactgatgagcgtttggctcgacaggaaaccgtgtggaatataacacctaagaatatgtctgttacccatgatatgatgctttttaaggccagccggggagaaaggactgtgtactctgtgtgttgggagggaggtggcaggttgaatactagggttctgtgagtttgattaaggtacggtgatcaatataagctatgtggtggtggggctatactactgaatgaaaaatgacttgaaattttctgcaattgaaaaataaacacgttgaaacataacatgcaacaggttcacgattctttattcctgggcaatgtaggagaaggtgtaagagttggtagcaaaagtttcagtggtgtattttccactttcccaggaccatgtaaaagacatagagtaagtgcttacctcgctagtttctgtggattcactagaa

SEQ ID NO: 18 - DNA, 743 bp, Adenovirus
  misc_feature 1..743: note = VA
  source 1..743: mol_type = genomic DNA
tcgatgtaggatgttgcccctcctgacgcggtaggagaaggggagggtgccctgcatgtctgccgctgctcttgctcttgccgctgctgaggaggggggcgcatctgccgcagcaccggatgcatctgggaaaagcaaaaaaggggctcgtccctgtttccggaggaatttgcaagcggggtcttgcatgacggggaggcaaacccccgttcgccgcagtccggccggcccgagactcgaaccgggggtcctgcgactcaacccttggaaaataaccctccggctacagggagcgagccacttaatgctttcgctttccagcctaaccgcttacgccgcgcgcggccagtggccaaaaaagctagcgcagcagccgccgcgcctggaaggaagccaaaaggagcgctcccccgttgtctgacgtcgcacacctgggttcgacacgcgggcggtaaccgcatggatcacggcggacggccggatccggggttcgaaccccggtcgtccgccatgatacccttgcgaatttatccaccagaccacggaagagtgcccgcttacaggctctccttttgcacggtctagagcgtcaacgactgcgcacgcctcaccggccagagcgtcccgaccatggagcactttttgccgctgcgcaacatctggaaccgcgtccgcgactttccgcgcgcctccaccaccgccgccggcatcacctggatgtccaggtacatctacggattacg